European Patent Specification EP 3 286 223 B1, published February 28, 2024. Title: KAPPA MYELOMA ANTIGEN CHIMERIC ANTIGEN RECEPTORS AND USES THEREOF. Applicant: HaemoLogiX Pty. Ltd. Micklethwaite, Kenneth Dunn, Rosanne Gottlieb, David Logan, Grant Harrison, Simon. The sequence listing filed with the application follows.

SEQUENCE LISTING (43 sequences)

SEQ ID NO: 1 - protein, 449 aa, Artificial Sequence
  human monoclonal antibody heavy chain
EVQLQQSGAELVKPGASVKLSCTASGFNIKDTYMHWVKQRPEQGLEWIGRIDPANGNTKYDPKFQGKATIIADTSSNTAYLQLSSLTSEDTAVYYCARGVYHDYDGDYWGQGTTLTVSSASTKGPSVFPLAPSSKSTSGGTAALGCLVKDYFPEPVTVSWNSGALTSGVHTFPAVLQSSGLYSLSSVVTVPSSSLGTQTYICNVNHKPSNTKVDKRVEPKSCDKTHTCPPCPAPELLGGPSVFLFPPKPKDTLMISRTPEVTCVVVDVSHEDPEVKFNWYVDGVEVHNAKTKPREEQYNSTYRVVSVLTVLHQDWLNGKEYKCKVSNKALPAPIEKTISKAKGQPREPQVYTLPPSREEMTKNQVSLTCLVKGFYPSDIAVEWESNGQPENNYKTTPPVLDSDGSFFLYSKLTVDKSRWQQGNVFSCSVMHEALHNHYTQKSLSLSPGK

SEQ ID NO: 2 - protein, 214 aa, Artificial Sequence
  human monoclonal antibody light chain
DIVMTQSQKFMSTSVGDRVSVTCKASQNVGTNVAWYQQKPGQSPKALIYSTSYRYSGVPDRFTGSGSGTDFTLTISNVQSEDLAEYFCQQYNSYPYTFGGGTKLEIKRTVAAPSVFIFPPSDEQLKSGTASVVCLLNNFYPREAKVQWKVDNALQSGNSQESVTEQDSKDSTYSLSSTLTLSKADYEKHKVYACEVTHQGLSSPVTKSFNRGEC

SEQ ID NO: 3 - protein, 5 aa, Artificial Sequence
  human monoclonal antibody VH CDR
DTYMH

SEQ ID NO: 4 - protein, 17 aa, Artificial Sequence
  human monoclonal antibody VH CDR
RIDPANGNTKYDPKFQG

SEQ ID NO: 5 - protein, 10 aa, Artificial Sequence
  human monoclonal antibody VH CDR
GVYHDYDGDY

SEQ ID NO: 6 - protein, 11 aa, Artificial Sequence
  human monoclonal antibody VL CDR
KASQNVGTNVA

SEQ ID NO: 7 - protein, 7 aa, Artificial Sequence
  human monoclonal antibody VL CDR
STSYRYS

SEQ ID NO: 8 - protein, 9 aa, Artificial Sequence
  human monoclonal antibody VL CDR
QQYNSYPYT

SEQ ID NO: 9 - DNA, 357 bp, Artificial Sequence
  human monoclonal antibody VH
gaggtgcagctgcagcagtcaggggcggagcttgtgaagccaggggcctcagtcaagttgtcctgtacagcttctggcttcaacattaaagacacctatatgcactgggtgaagcagaggcctgaacagggcctggagtggattggaaggattgatcctgcgaatggtaacactaaatatgacccgaagttccagggcaaggccactataatagcagacacatcctccaacacagcctacctgcagctcagcagcctgacatctgaggacactgccgtctattactgtgctaggggggtctaccatgattacgacggggactactggggccaagggaccacgctcaccgtctcctcc

SEQ ID NO: 10 - DNA, 321 bp, Artificial Sequence
  human monoclonal antibody VL
gacatcgtcatgacccagtctcaaaaattcatgtccacatcagtaggagacagggtcagcgtcacctgcaaggccagtcagaatgtgggtactaatgtagcctggtatcaacagaaaccagggcaatctcctaaagcactgatttactcgacatcctaccggtacagtggagtccctgatcgcttcacaggcagtggatctgggacagatttcactctcaccatcagcaatgtgcagtctgaagacttggcagagtatttctgtcagcaatataacagctatccgtacacgttcggaggggggaccaagctggaaataaag

SEQ ID NO: 11 - DNA, 1200 bp, Artificial Sequence
  human monoclonal antibody VH DNA in pHCMV-Gamm1-neo expression vector
  misc_feature (11)..(11): n is a, c, g, or t
  misc_feature (947)..(947): n is a, c, g, or t
  misc_feature (998)..(998): n is a, c, g, or t
  misc_feature (1009)..(1009): n is a, c, g, or t
  misc_feature (1027)..(1027): n is a, c, g, or t
  misc_feature (1032)..(1032): n is a, c, g, or t
  misc_feature (1036)..(1036): n is a, c, g, or t
  misc_feature (1044)..(1044): n is a, c, g, or t
  misc_feature (1065)..(1065): n is a, c, g, or t
  misc_feature (1085)..(1085): n is a, c, g, or t
  misc_feature (1095)..(1095): n is a, c, g, or t
  misc_feature (1099)..(1100): n is a, c, g, or t
  misc_feature (1105)..(1105): n is a, c, g, or t
  misc_feature (1108)..(1108): n is a, c, g, or t
  misc_feature (1111)..(1111): n is a, c, g, or t
  misc_feature (1127)..(1127): n is a, c, g, or t
  misc_feature (1134)..(1134): n is a, c, g, or t
  misc_feature (1136)..(1136): n is a, c, g, or t
  misc_feature (1157)..(1157): n is a, c, g, or t
  misc_feature (1168)..(1168): n is a, c, g, or t
  misc_feature (1172)..(1172): n is a, c, g, or t
  misc_feature (1190)..(1190): n is a, c, g, or t
caggacgatcngcctccgcaagcttatgaatatgcaaatcctctgaatctacatggtaaatataggtttgtctataccacaaacagaaaaacatgagatcacagttctctctacagttactgagcacacaggacctcaccatgggatggagctgtatcatcctcttcttggtagcaacagctacaggtaaggggctcacagtagcaggcttgaggtctggacatatatatgggtgacaatgacatccactttgcctttctctccacaggtgtgcactccgaggtgcagctgcagcagtcaggggcggagcttgtgaagccaggggcctcagtcaagttgtcctgtacagcttctggcttcaacattaaagacacctatatgcactgggtgaagcagaggcctgaacagggcctggagtggattggaaggattgatcctgcgaatggtaacactaaatatgacccgaagttccagggcaaggccactataatagcagacacatcctccaacacagcctacctgcagctcagcagcctgacatctgaggacactgccgtctattactgtgctaggggggtctaccatgattacgacggggactactggggccaagggaccacgctcaccgtctcctccggtgagtggatcccaagctagctttctggggcaggccaggcctgaccttggctttggggcagggagggggctaaggtgaggcaggtggcgccagccaggtgcacacccaatgcccatgagcccagacactggacgctgaacctcgcggacagttaagaacccaggggcctctgcgccctgggcccagctctgtcccacaccgcggtcacatggcaccacctctcttgcagcctccaccaagggcccatcggtcttccccctggcacccctcctccaagagcacctctgggggcacagcggccctgggctgncctggtcaaggactacttcccccgaaccggtgacggtgtcgtggaactcangcgccctgacnagcggggtgcacaccttnccggntgtnctacagtnctcaggactctactccctcancagcgtggtgaccgtgcccntcagcagctngggnncccanacntanatttgcacgggaatcnaagcccngnaacccaaggggaaaaaaaaanttggtgaaagncccnccagggagggaggggttntgctggaaac

SEQ ID NO: 12 - DNA, 1121 bp, Artificial Sequence
  human monoclonal antibody VL DNA in pHCMV-Gamm1-neo expression vector
  misc_feature (1)..(1): n is a, c, g, or t
  misc_feature (12)..(12): n is a, c, g, or t
  misc_feature (983)..(983): n is a, c, g, or t
  misc_feature (1002)..(1003): n is a, c, g, or t
  misc_feature (1014)..(1014): n is a, c, g, or t
  misc_feature (1055)..(1055): n is a, c, g, or t
  misc_feature (1057)..(1057): n is a, c, g, or t
  misc_feature (1084)..(1084): n is a, c, g, or t
  misc_feature (1092)..(1092): n is a, c, g, or t
  misc_feature (1098)..(1098): n is a, c, g, or t
  misc_feature (1110)..(1110): n is a, c, g, or t
  misc_feature (1113)..(1113): n is a, c, g, or t
  misc_feature (1119)..(1119): n is a, c, g, or t
  misc_feature (1121)..(1121): n is a, c, g, or t
ncagggcgatcngcctccgcaagcttatgaatatgcaaatcctctgaatctacatggtaaatataggtttgtctataccacaaacagaaaaacatgagatcacagttctctctacagttactgagcacacaggacctcaccatgggatggagctgtatcatcctcttcttggtagcaacagctacaggtaaggggctcacagtagcaggcttgaggtctggacatatatatgggtgacaatgacatccactttgcctttctctccacaggtgtgcactccgacatcgtcatgacccagtctcaaaaattcatgtccacatcagtaggagacagggtcagcgtcacctgcaaggccagtcagaatgtgggtactaatgtagcctggtatcaacagaaaccagggcaatctcctaaagcactgatttactcgacatcctaccggtacagtggagtccctgatcgcttcacaggcagtggatctgggacagatttcactctcaccatcagcaatgtgcagtctgaagacttggcagagtatttctgtcagcaatataacagctatccgtacacgttcggaggggggaccaagctggaaataaagggtgagtggatcctagaattctaaactctgagggggtcggatgacgtggccattctttgcctaaagcattgagtttactgcaaggtcagaaaagcatgcaaagccctcagaatggctgcaaagagctccaacaaaacaatttagaactttattaaggaatagggggaagctaggaagaaactcaaaacatcaagattttaaatacgcttcttggtctccttgctataattatctgggataagcatgctgttttctgtctgtccctaacatgccctgtgattatccgcaaacaacacacccaagggcagaactttgttacttaaacaccatcctgtttgcttctttcctcaggaactgtggctgcaccatctgtcttcatctncccgccatctgatgagcanntgaaatctggnaactgcctctgttgtgtgcctgctgaaaaacttctatcccnanaggccaaagtacagtggaaggggaaanccccctcnatcggnaactcccggaanggncccgancn

SEQ ID NO: 13 - DNA, 15 bp, Artificial Sequence
  human monoclonal antibody VH CDR
gacacctatatgcac

SEQ ID NO: 14 - DNA, 51 bp, Artificial Sequence
  human monoclonal antibody VH CDR
aggattgatcctgcgaatggtaacactaaatatgacccgaagttccagggc

SEQ ID NO: 15 - DNA, 30 bp, Artificial Sequence
  human monoclonal antibody VH CDR
ggggtctaccatgattacgacggggactac

SEQ ID NO: 16 - DNA, 33 bp, Artificial Sequence
  human monoclonal antibody VL CDR
aaggccagtcagaatgtgggtactaatgtagcc

SEQ ID NO: 17 - DNA, 21 bp, Artificial Sequence
  human monoclonal antibody VL CDR
tcgacatcctaccggtacagt

SEQ ID NO: 18 - DNA, 27 bp, Artificial Sequence
  human monoclonal antibody VL CDR
cagcaatataacagctatccgtacacg

SEQ ID NO: 19 - protein, 530 aa, Artificial Sequence
  Flexi-IL12
MCHQQLVISWFSLVFLASPLVAIWELKKDVYVVELDWYPDAPGEMVVLTCDTPEEDGITWTLDQSSEVLGSGKTLTIQVKEFGDAGQYTCHKGGEVLSHSLLLLHKKEDGIWSTDILKDQKEPKNKTFLRCEAKNYSGRFTCWWLTTISTDLTFSVKSSRGSSDPQGVTCGAATLSAERVRGDNKEYEYSVECQEDSACPAAEESLPIEVMVDAVHKLKYENYTSSFFIRDIIKPDPPKNLQLKPLKNSRQVEVSWEYPDTWSTPHSYFSLTFCVQVQGKSKREKKDRVFTDKTSATVICRKNASISVRAQDRYYSSSWSEWASVPCSGGGGSGGGGSGGGGSRNLPVATPDPGMFPCLHHSQNLLRAVSNMLQKARQTLEFYPCTSEEIDHEDITKDKTSTVEACLPLELTKNESCLNSRETSFITNGSCLASRKTSFMMALCLSSIYEDLKMYQVEFKTMNAKLLMDPKRQIFLDQNMLAVIDELMQALNFNSETVPQKSSLEEPDFYKAFRIRAVTIDRVMSYLNAS

SEQ ID NO: 20 - protein, 21 aa, Artificial Sequence
  IgG heavy chain leader component of KM.CAR-hCH2CH3-28z construct
MEFGLSWLFLVAILKGVQCSR

SEQ ID NO: 21 - protein, 107 aa, Artificial Sequence
  KappaMab variable light chain component of KM.CAR-hCH2CH3-28z construct
DIVMTQSQKFMSTSVGDRVSVTCKASQNVGTNVAWYQQKPGQSPKALIYSTSYRYSGVPDRFTGSGSGTDFTLTISNVQSEDLAEYFCQQYNSYPYTFGGGTKLEIK

SEQ ID NO: 22 - skipped
  KappaMab variable heavy chain component of KM.CAR-hCH2CH3-28z construct

SEQ ID NO: 23 - protein, 15 aa, Artificial Sequence
  (G4S)3 flexible linker component of KM.CAR-hCH2CH3-28z construct
GGGGSGGGGSGGGGS

SEQ ID NO: 24 - protein, 246 aa, Artificial Sequence
  Hinge, CH2 and CH3 components of KM.CAR-hCH2CH3-28z construct
YVTVSSQDPAEPKSPDKTHTCPPCPAPELLGGPSVFLFPPKPKDTLMISRTPEVTCVVVDVSHEDPEVKFNWYVDGVEVHNAKTKPREEQYNSTYRVVSVLTVLHQDWLNGKEYKCKVSNKALPAPIEKTISKAKGQPREPQVYTLPPSRDELTKNQVSLTCLVKGFYPSDIAVEWESNGQPENNYKTTPPVLDSDGSFFLYSKLTVDKSRWQQGNVFSCSVMHEALHNHYTQKSLSLSPGKKDPK

SEQ ID NO: 25 - protein, 68 aa, Homo sapiens
FWVLVVVGGVLACYSLLVTVAFIIFWVRSKRSRLLHSDYMNMTPRRPGPTRKHYQPYAPPRDFAAYRS

SEQ ID NO: 26 - protein, 112 aa, Homo sapiens
RVKFSRSADAPAYQQGQNQLYNELNLGRREEYDVLDKRRGRDPEMGGKPRRKNPQEGLYNELQKDKMAEAYSEIGMKGERRRGKGHDGLYQGLSTATKDTYDALHMQALPPR

SEQ ID NO: 27 - protein, 688 aa, Artificial Sequence
  Full length KM.CAR-hCH2CH3-28z amino acid construct
MEFGLSWLFLVAILKGVQCSRDIVMTQSQKFMSTSVGDRVSVTCKASQNVGTNVAWYQQKPGQSPKALIYSTSYRYSGVPDRFTGSGSGTDFTLTISNVQSEDLAEYFCQQYNSYPYTFGGGTKLEIKGGGGSGGGGSGGGGSEVQLQQSGAELVKPGASVKLSCTASGFNIKDTYMHWVKQRPEQGLEWIGRIDPANGNTKYDPKFQGKATIIADTSSNTAYLQLSSLTSEDTAVYYCARGVYHDYDGDYWGQGTTLTVSSYVTVSSQDPAEPKSPDKTHTCPPCPAPELLGGPSVFLFPPKPKDTLMISRTPEVTCVVVDVSHEDPEVKFNWYVDGVEVHNAKTKPREEQYNSTYRVVSVLTVLHQDWLNGKEYKCKVSNKALPAPIEKTISKAKGQPREPQVYTLPPSRDELTKNQVSLTCLVKGFYPSDIAVEWESNGQPENNYKTTPPVLDSDGSFFLYSKLTVDKSRWQQGNVFSCSVMHEALHNHYTQKSLSLSPGKKDPKFWVLVVVGGVLACYSLLVTVAFIIFWVRSKRSRLLHSDYMNMTPRRPGPTRKHYQPYAPPRDFAAYRSRVKFSRSADAPAYQQGQNQLYNELNLGRREEYDVLDKRRGRDPEMGGKPRRKNPQEGLYNELQKDKMAEAYSEIGMKGERRRGKGHDGLYQGLSTATKDTYDALHMQALPPR

SEQ ID NO: 28 - DNA, 2064 bp, Artificial Sequence
  Full length KM.CAR-hCH2CH3-28z nucleic acid construct
atggagtttgggctgagctggctttttcttgtggctattttaaaaggtgtccagtgctctagagacatcgtcatgacccagtctcaaaaattcatgtccacatcagtaggagacagggtcagcgtcacctgcaaggccagtcagaatgtgggtactaatgtagcctggtatcaacagaaaccagggcaatctcctaaagcactgatttactcgacatcctaccggtacagtggagtccctgatcgcttcacaggcagtggatctgggacagatttcactctcaccatcagcaatgtgcagtctgaagacttggcagagtatttctgtcagcaatataacagctatccgtacacgttcggaggggggaccaagctggaaataaagggtggcggtggctcgggcggtggtgggtcgggtggcggcggatctgaggtgcagctgcagcagtcaggggcggagcttgtgaagccaggggcctcagtcaagttgtcctgtacagcttctggcttcaacattaaagacacctatatgcactgggtgaagcagaggcctgaacagggcctggagtggattggaaggattgatcctgcgaatggtaacactaaatatgacccgaagttccagggcaaggccactataatagcagacacatcctccaacacagcctacctgcagctcagcagcctgacatctgaggacactgccgtctattactgtgctaggggggtctaccatgattacgacggggactactggggccaagggaccacgctcaccgtctcctcctacgtcaccgtctcttcacaggatcccgccgagcccaaatctcctgacaaaactcacacatgcccaccgtgcccagcacctgaactcctggggggaccgtcagtcttcctcttccccccaaaacccaaggacaccctcatgatctcccggacccctgaggtcacatgcgtggtggtggacgtgagccacgaagaccctgaggtcaagttcaactggtacgtggacggcgtggaggtgcataatgccaagacaaagccgcgggaggagcagtacaacagcacgtaccgtgtggtcagcgtcctcaccgtcctgcaccaggactggctgaatggcaaggagtacaagtgcaaggtctccaacaaagccctcccagcccccatcgagaaaaccatctccaaagccaaagggcagccccgagaaccacaggtgtacaccctgcccccatcccgggatgagctgaccaagaaccaggtcagcctgacctgcctggtcaaaggcttctatcccagcgacatcgccgtggagtgggagagcaatgggcaaccggagaacaactacaagaccacgcctcccgtgctggactccgacggctccttcttcctctacagcaagctcaccgtggacaagagcaggtggcagcaggggaacgtcttctcatgctccgtgatgcatgaggctctgcacaaccactacacgcagaagagcctctccctgtctccgggtaaaaaagatcccaaattttgggtgctggtggtggttggtggagtcctggcttgctatagcttgctagtaacagtggcctttattattttctgggtgaggagtaagaggagcaggctcctgcacagtgactacatgaacatgactccccgccgccccgggcccacccgcaagcattaccagccctatgccccaccacgcgacttcgcagcctatcgctccagagtgaagttcagcaggagcgcagacgcccccgcgtaccagcagggccagaaccagctctataacgagctcaatctaggacgaagagaggagtacgatgttttggacaagagacgtggccgggaccctgagatggggggaaagccgagaaggaagaaccctcaggaaggcctgtacaatgaactgcagaaagataagatggcggaggcctacagtgagattgggatgaaaggcgagcgccggaggggcaaggggcacgatggcctttaccagggtctcagtacagccaccaaggacacctacgacgcccttcacatgcaggccctgccccctcgc

SEQ ID NO: 29 - DNA, 1727 bp, Artificial Sequence
  Full length KM.CAR-hCH3-28z nucleic acid construct
tggagtttgggctgagctggctttttcttgtggctattttaaaaggtgtccagtgctctagagacatcgtcatgacccagtctcaaaaattcatgtccacatcagtaggagacagggtcagcgtcacctgcaaggccagtcagaatgtgggtactaatgtagcctggtatcaacagaaaccagggcaatctcctaaagcactgatttactcgacatcctaccggtacagtggagtccctgatcgcttcacaggcagtggatctgggacagatttcactctcaccatcagcaatgtgcagtctgaagacttggcagagtatttctgtcagcaatataacagctatccgtacacgttcggaggggggaccaagctggaaataaagggtggcggtggctcgggcggtggtgggtcgggtggcggcggatctgaggtgcagctgcagcagtcaggggcggagcttgtgaagccaggggcctcagtcaagttgtcctgtacagcttctggcttcaacattaaagacacctatatgcactgggtgaagcagaggcctgaacagggcctggagtggattggaaggattgatcctgcgaatggtaacactaaatatgacccgaagttccagggcaaggccactataatagcagacacatcctccaacacagcctacctgcagctcagcagcctgacatctgaggacactgccgtctattactgtgctaggggggtctaccatgattacgacggggactactggggccaagggaccacgctcaccgtctcctccggtggaggcgggtctgggggcggaggttcaggcgggggtggttccgagcccaaatctcctgacaaaactcacacatgcccagggcagccccgagaaccacaggtgtacaccctgcccccatcccgggatgagctgaccaagaaccaggtcagcctgacctgcctggtcaaaggcttctatcccagcgacatcgccgtggagtgggagagcaatgggcagccggagaacaactacaagaccacgcctcccgtgctggactccgacggctccttcttcctctacagcaagctcaccgtggacaagagcaggtggcagcaggggaacgtcttctcatgctccgtgatgcatgaggctctgcacaaccactacacacagaagagcctctccctgtctccgggtaaattttgggtgctggtggtggttggtggagtcctggcttgctatagcttgctagtaacagtggcctttattattttctgggtgaggagtaagaggagcaggctcctgcacagtgactacatgaacatgactccccgccgccccgggcccacccgcaagcattaccagccctatgccccaccacgcgacttcgcagcctatcgctccagagtgaagttcagcaggagcgcagacgcccccgcgtaccagcagggccagaaccagctctataacgagctcaatctaggacgaagagaggagtacgatgttttggacaagagacgtggccgggaccctgagatggggggaaagccgagaaggaagaaccctcaggaaggcctgtacaatgaactgcagaaagataagatggcggaggcctacagtgagattgggatgaaaggcgagcgccggaggggcaaggggcacgatggcctttaccagggtctcagtacagccaccaaggacacctacgacgcccttcacatgcaggccctgccccctcgc

SEQ ID NO: 30 - DNA, 1407 bp, Artificial Sequence
  Full length KM.CAR-h-28z nucleic acid construct
atggagtttgggctgagctggctttttcttgtggctattttaaaaggtgtccagtgctctagagacatcgtcatgacccagtctcaaaaattcatgtccacatcagtaggagacagggtcagcgtcacctgcaaggccagtcagaatgtgggtactaatgtagcctggtatcaacagaaaccagggcaatctcctaaagcactgatttactcgacatcctaccggtacagtggagtccctgatcgcttcacaggcagtggatctgggacagatttcactctcaccatcagcaatgtgcagtctgaagacttggcagagtatttctgtcagcaatataacagctatccgtacacgttcggaggggggaccaagctggaaataaagggtggcggtggctcgggcggtggtgggtcgggtggcggcggatctgaggtgcagctgcagcagtcaggggcggagcttgtgaagccaggggcctcagtcaagttgtcctgtacagcttctggcttcaacattaaagacacctatatgcactgggtgaagcagaggcctgaacagggcctggagtggattggaaggattgatcctgcgaatggtaacactaaatatgacccgaagttccagggcaaggccactataatagcagacacatcctccaacacagcctacctgcagctcagcagcctgacatctgaggacactgccgtctattactgtgctaggggggtctaccatgattacgacggggactactggggccaagggaccacgctcaccgtctcctccggtggaggcgggtctgggggcggaggttcaggcgggggtggttccgagcccaaatctcctgacaaaactcacacatgcccattttgggtgctggtggtggttggtggagtcctggcttgctatagcttgctagtaacagtggcctttattattttctgggtgaggagtaagaggagcaggctcctgcacagtgactacatgaacatgactccccgccgccccgggcccacccgcaagcattaccagccctatgccccaccacgcgacttcgcagcctatcgctccagagtgaagttcagcaggagcgcagacgcccccgcgtaccagcagggccagaaccagctctataacgagctcaatctaggacgaagagaggagtacgatgttttggacaagagacgtggccgggaccctgagatggggggaaagccgagaaggaagaaccctcaggaaggcctgtacaatgaactgcagaaagataagatggcggaggcctacagtgagattgggatgaaaggcgagcgccggaggggcaaggggcacgatggcctttaccagggtctcagtacagccaccaaggacacctacgacgcccttcacatgcaggccctgccccctcgc

SEQ ID NO: 31 - DNA, 1461 bp, Artificial Sequence
  Full length KM.CAR-CD8a-28z nucleic acid construct
atggagtttgggctgagctggctttttcttgtggctattttaaaaggtgtccagtgctctagagacatcgtcatgacccagtctcaaaaattcatgtccacatcagtaggagacagggtcagcgtcacctgcaaggccagtcagaatgtgggtactaatgtagcctggtatcaacagaaaccagggcaatctcctaaagcactgatttactcgacatcctaccggtacagtggagtccctgatcgcttcacaggcagtggatctgggacagatttcactctcaccatcagcaatgtgcagtctgaagacttggcagagtatttctgtcagcaatataacagctatccgtacacgttcggaggggggaccaagctggaaataaagggtggcggtggctcgggcggtggtgggtcgggtggcggcggatctgaggtgcagctgcagcagtcaggggcggagcttgtgaagccaggggcctcagtcaagttgtcctgtacagcttctggcttcaacattaaagacacctatatgcactgggtgaagcagaggcctgaacagggcctggagtggattggaaggattgatcctgcgaatggtaacactaaatatgacccgaagttccagggcaaggccactataatagcagacacatcctccaacacagcctacctgcagctcagcagcctgacatctgaggacactgccgtctattactgtgctaggggggtctaccatgattacgacggggactactggggccaagggaccacgctcaccgtctcctccaccacgacgccagcgccgcgaccaccaacaccggcgcccaccatcgcgtcgcagcccctgtccctgcgcccagaggcgtgccggccagcggcggggggcgcagtgcacacgagggggctggacttcgcctgtgatttttgggtgctggtggtggttggtggagtcctggcttgctatagcttgctagtaacagtggcctttattattttctgggtgaggagtaagaggagcaggctcctgcacagtgactacatgaacatgactccccgccgccccgggcccacccgcaagcattaccagccctatgccccaccacgcgacttcgcagcctatcgctccagagtgaagttcagcaggagcgcagacgcccccgcgtaccagcagggccagaaccagctctataacgagctcaatctaggacgaagagaggagtacgatgttttggacaagagacgtggccgggaccctgagatggggggaaagccgagaaggaagaaccctcaggaaggcctgtacaatgaactgcagaaagataagatggcggaggcctacagtgagattgggatgaaaggcgagcgccggaggggcaaggggcacgatggcctttaccagggtctcagtacagccaccaaggacacctacgacgcccttcacatgcaggccctgccccctcgc

SEQ ID NO: 32 - DNA, 1410 bp, Artificial Sequence
  Full length KM.CAR-h-28TM-41BBz nucleic acid construct
atggagtttgggctgagctggctttttcttgtggctattttaaaaggtgtccagtgctctagagacatcgtcatgacccagtctcaaaaattcatgtccacatcagtaggagacagggtcagcgtcacctgcaaggccagtcagaatgtgggtactaatgtagcctggtatcaacagaaaccagggcaatctcctaaagcactgatttactcgacatcctaccggtacagtggagtccctgatcgcttcacaggcagtggatctgggacagatttcactctcaccatcagcaatgtgcagtctgaagacttggcagagtatttctgtcagcaatataacagctatccgtacacgttcggaggggggaccaagctggaaataaagggtggcggtggctcgggcggtggtgggtcgggtggcggcggatctgaggtgcagctgcagcagtcaggggcggagcttgtgaagccaggggcctcagtcaagttgtcctgtacagcttctggcttcaacattaaagacacctatatgcactgggtgaagcagaggcctgaacagggcctggagtggattggaaggattgatcctgcgaatggtaacactaaatatgacccgaagttccagggcaaggccactataatagcagacacatcctccaacacagcctacctgcagctcagcagcctgacatctgaggacactgccgtctattactgtgctaggggggtctaccatgattacgacggggactactggggccaagggaccacgctcaccgtctcctccggtggaggcgggtctgggggcggaggttcaggcgggggtggttccgagcccaaatctcctgacaaaactcacacatgcccattttgggtgctggtggtggttggtggagtcctggcttgctatagcttgctagtaacagtggcctttattattttctgggtgaaacggggcagaaagaaactcctgtatatattcaaacaaccatttatgagaccagtacaaactactcaagaggaagatggctgtagctgccgatttccagaagaagaagaaggaggatgtgaactgagagtgaagttcagcaggagcgcagacgcccccgcgtaccagcagggccagaaccagctctataacgagctcaatctaggacgaagagaggagtacgatgttttggacaagagacgtggccgggaccctgagatggggggaaagccgagaaggaagaaccctcaggaaggcctgtacaatgaactgcagaaagataagatggcggaggcctacagtgagattgggatgaaaggcgagcgccggaggggcaaggggcacgatggcctttaccagggtctcagtacagccaccaaggacacctacgacgcccttcacatgcaggccctgccccctcgc

SEQ ID NO: 33 - DNA, 1464 bp, Artificial Sequence
  Full length KM.CAR_8a_28TM_41BBz nucleic acid construct
atggagtttgggctgagctggctttttcttgtggctattttaaaaggtgtccagtgctctagagacatcgtcatgacccagtctcaaaaattcatgtccacatcagtaggagacagggtcagcgtcacctgcaaggccagtcagaatgtgggtactaatgtagcctggtatcaacagaaaccagggcaatctcctaaagcactgatttactcgacatcctaccggtacagtggagtccctgatcgcttcacaggcagtggatctgggacagatttcactctcaccatcagcaatgtgcagtctgaagacttggcagagtatttctgtcagcaatataacagctatccgtacacgttcggaggggggaccaagctggaaataaagggtggcggtggctcgggcggtggtgggtcgggtggcggcggatctgaggtgcagctgcagcagtcaggggcggagcttgtgaagccaggggcctcagtcaagttgtcctgtacagcttctggcttcaacattaaagacacctatatgcactgggtgaagcagaggcctgaacagggcctggagtggattggaaggattgatcctgcgaatggtaacactaaatatgacccgaagttccagggcaaggccactataatagcagacacatcctccaacacagcctacctgcagctcagcagcctgacatctgaggacactgccgtctattactgtgctaggggggtctaccatgattacgacggggactactggggccaagggaccacgctcaccgtctcctccaccacgacgccagcgccgcgaccaccaacaccggcgcccaccatcgcgtcgcagcccctgtccctgcgcccagaggcgtgccggccagcggcggggggcgcagtgcacacgagggggctggacttcgcctgtgatttttgggtgctggtggtggttggtggagtcctggcttgctatagcttgctagtaacagtggcctttattattttctgggtgaaacggggcagaaagaaactcctgtatatattcaaacaaccatttatgagaccagtacaaactactcaagaggaagatggctgtagctgccgatttccagaagaagaagaaggaggatgtgaactgagagtgaagttcagcaggagcgcagacgcccccgcgtaccagcagggccagaaccagctctataacgagctcaatctaggacgaagagaggagtacgatgttttggacaagagacgtggccgggaccctgagatggggggaaagccgagaaggaagaaccctcaggaaggcctgtacaatgaactgcagaaagataagatggcggaggcctacagtgagattgggatgaaaggcgagcgccggaggggcaaggggcacgatggcctttaccagggtctcagtacagccaccaaggacacctacgacgcccttcacatgcaggccctgccccctcgc

SEQ ID NO: 34 - DNA, 2067 bp, Artificial Sequence
  Full length KM.CAR_hCH2CH3mut_28TM_41BBz nucleic acid construct
atggagtttgggctgagctggctttttcttgtggctattttaaaaggtgtccagtgctctagagacatcgtcatgacccagtctcaaaaattcatgtccacatcagtaggagacagggtcagcgtcacctgcaaggccagtcagaatgtgggtactaatgtagcctggtatcaacagaaaccagggcaatctcctaaagcactgatttactcgacatcctaccggtacagtggagtccctgatcgcttcacaggcagtggatctgggacagatttcactctcaccatcagcaatgtgcagtctgaagacttggcagagtatttctgtcagcaatataacagctatccgtacacgttcggaggggggaccaagctggaaataaagggtggcggtggctcgggcggtggtgggtcgggtggcggcggatctgaggtgcagctgcagcagtcaggggcggagcttgtgaagccaggggcctcagtcaagttgtcctgtacagcttctggcttcaacattaaagacacctatatgcactgggtgaagcagaggcctgaacagggcctggagtggattggaaggattgatcctgcgaatggtaacactaaatatgacccgaagttccagggcaaggccactataatagcagacacatcctccaacacagcctacctgcagctcagcagcctgacatctgaggacactgccgtctattactgtgctaggggggtctaccatgattacgacggggactactggggccaagggaccacgctcaccgtctcctccggtggaggcgggtctgggggcggaggttcaggcgggggtggttccgagcccaaatctcctgacaaaactcacacatgcccaccgtgcccagcacctccagtcgcgggaccgtcagtcttcctcttccccccaaaacccaaggacaccctcatgatcgcccggacccctgaggtcacatgcgtggtggtgaacgtgagccacgaagaccctgaggtcaagttcaactggtacgtggacggcgtggaggtgcataatgccaagacaaagccgcgggaggagcagtacgccagcacgtaccgtgtggtcagcgtcctcaccgtcctgcaccaggactggctgaatggcaaggagtacaagtgcaaggtctccaacaaagccctcccagcccccatcgagaaaaccatctccaaagccaaagggcagccccgagaaccacaggtgtacaccctgcccccatcccgggatgagctgaccaagaaccaggtcagcctgacctgcctggtcaaaggcttctatcccagcgacatcgccgtggagtgggagagcaatgggcagccggagaacaactacaagaccacgcctcccgtgctggactccgacggctccttcttcctctacagcaagctcaccgtggacaagagcaggtggcagcaggggaacgtcttctcatgctccgtgatgcatgaggctctgcacaaccactacacacagaagagcctctccctgtctccgggtaaattttgggtgctggtggtggttggtggagtcctggcttgctatagcttgctagtaacagtggcctttattattttctgggtgaaacggggcagaaagaaactcctgtatatattcaaacaaccatttatgagaccagtacaaactactcaagaggaagatggctgtagctgccgatttccagaagaagaagaaggaggatgtgaactgagagtgaagttcagcaggagcgcagacgcccccgcgtaccagcagggccagaaccagctctataacgagctcaatctaggacgaagagaggagtacgatgttttggacaagagacgtggccgggaccctgagatggggggaaagccgagaaggaagaaccctcaggaaggcctgtacaatgaactgcagaaagataagatggcggaggcctacagtgagattgggatgaaaggcgagcgccggaggggcaaggggcacgatggcctttaccagggtctcagtacagccaccaaggacacctacgacgcccttcacatgcaggccctgccccctcgc

SEQ ID NO: 35 - DNA, 30 bp, Homo sapiens
ggaggaaaaactgtttcatacagaaggcgt

SEQ ID NO: 36 - DNA, 114 bp, Homo sapiens
acattttgacacccccataatatttttccagaattaacagtataaattgcatctcttgttcaagagttccctatcactctctttaatcactactcacagtaacctcaactcctg

SEQ ID NO: 37 - DNA, 1233 bp, Artificial Sequence
  Constructed nucleic acid sequence of transposon gene expression cassette
ggaggaaaaactgtttcatacagaaggcgtcaattaggaggaaaaactgtttcatacagaaggcgtcaattaggaggaaaaactgtttcatacagaaggcgtcaattgtcccatcgaattaggaggaaaaactgtttcatacagaaggcgtcaattaggaggaaaaactgtttcatacagaaggcgtcaattaggaggaaaaactgtttcatacagaaggcgtcaattgtcccgggacattttgacacccccataatatttttccagaattaacagtataaattgcatctcttgttcaagagttccctatcactctctttaatcactactcacagtaacctcaactcctgaactccatggatggtgagcaagggcgaggagctgttcaccggggtggtgcccatcctggtcgagctggacggcgacgtaaacggccacaagttcagcgtgtccggcgagggcgagggcgatgccacctacggcaagctgaccctgaagttcatctgcaccaccggcaagctgcccgtgccctggcccaccctcgtgaccaccctgacctacggcgtgcagtgcttcagccgctaccccgaccacatgaagcagcacgacttcttcaagtccgccatgcccgaaggctacgtccaggagcgcaccatcttcttcaaggacgacggcaactacaagacccgcgccgaggtgaagttcgagggcgacaccctggtgaaccgcatcgagctgaagggcatcgacttcaaggaggacggcaacatcctggggcacaagctggagtacaactacaacagccacaacgtctatatcatggccgacaagcagaagaacggcatcaaggtgaacttcaagatccgccacaacatcgaggacggcagcgtgcagctcgccgaccactaccagcagaacacccccatcggatccggagccacgaacttctctctgttaaagcaagcaggagacgttgaagaaaaccccggtcctatttaaatcctcgactgtgccttctagttgccagccatctgttgtttgcccctcccccgtgccttccttgaccctggaaggtgccactcccactgtcctttcctaataaaatgaggaaattgcatcgcattgtctgagtaggtgtcattctattctggggggtggggtggggcaggacagcaagggggaggattgggaagacaatagcaggcatgctggggatgcggtgggctctatggc

SEQ ID NO: 38 - protein, 218 aa, Artificial Sequence
  Mutated SANT-7 amino acid sequence
MNSFSTSAFGPVAFSLGLLLVLPAAFPAPVPPGEDSKDVAAPHRQPLTSSERIDKQIRDILDFISALRKETCNKSNMCESSKEADAFWNLNLPKMAEKDGCFYKGFNEETCLVKIITGLLEFEVYLEYLQNRFESSEEQARAVQMRTKDLIQFLQKKAKNLDAITTPDPTTNASLLTKLQAQNQWLQDMTTHLILRSFKEFLIRSLRALRAMHHHHHH

SEQ ID NO: 39 - DNA, 655 bp, Artificial Sequence
  Mutated SANT-7 nucleic acid sequence
atgaactccttctccacaagcgccttcggtccagttgccttctccctggggctgctcctggtgttgcctgctgccttccctgccccagtacccccaggagaagattccaaagatgtagccgccccacacagacagccactcacgagctcagaacgaattgacaaacaaattcgggacatcctcgactttatctcagccttaagaaaggagacatgtaacaagagtaacatgtgtgagagctccaaagaggcagacgcattctggaacctgaaccttccaaagatggctgaaaaagatggatgcttctacaaaggattcaatgaggagacttgcctggtgaaaatcatcactggtcttctcgagtttgaggtatacctagagtacctccagaacagatttgagagtagtgaggaacaagccagagctgtgcagatgcgcacaaaagacctgatccagttcctgcagaaaaaggcaaagaatctagatgcaataaccacccctgacccaaccacaaatgccagcctgctgacgaagctgcaggcacagaaccagtggctgcaggacatgacaactcatctcattctgagatcttttaaggagttcctgatccgtagcctgagggctcttcgggctatgcatcatcaccatcaccact

SEQ ID NO: 40 - protein, 540 aa, Artificial Sequence
  Flexi-IL-12 amino acid construct
MCHQQLVISWFSLVFLASPLVAIWELKKDVYVVELDWYPDAPGEMVVLTCDTPEEDGITWTLDQSSEVLGSGKTLTIQVKEFGDAGQYTCHKGGEVLSHSLLLLHKKEDGIWSTDILKDQKEPKNKTFLRCEAKNYSGRFTCWWLTTISTDLTFSVKSSRGSSDPQGVTCGAATLSAERVRGDNKEYEYSVECQEDSACPAAEESLPIEVMVDAVHKLKYENYTSSFFIRDIIKPDPPKNLQLKPLKNSRQVEVSWEYPDTWSTPHSYFSLTFCVQVQGKSKREKKDRVFTDKTSATVICRKNASISVRAQDRYYSSSWSEWASVPCSGGGGSGGGGSGGGGSRNLPVATPDPGMFPCLHHSQNLLRAVSNMLQKARQTLEFYPCTSEEIDHEDITKDKTSTVEACLPLELTKNESCLNSRETSFITNGSCLASRKTSFMMALCLSSIYEDLKMYQVEFKTMNAKLLMDPKRQIFLDQNMLAVIDELMQALNFNSETVPQKSSLEEPDFYKTKIKLCILLHAFRIRAVTIDRVMSYLNAS

SEQ ID NO: 41 - DNA, 1620 bp, Artificial Sequence
  Flexi-IL-12 nucleic acid construct
atgtgtcaccagcagttggtcatctcttggttttccctggtttttctggcatctcccctcgtggccatatgggaactgaagaaagatgtttatgtcgtagaattggattggtatccggatgcccctggagaaatggtggtcctcacctgtgacacccctgaagaagatggtatcacctggaccttggaccagagcagtgaggtcttaggctctggcaaaaccctgaccatccaagtcaaagagtttggagatgctggccagtacacctgtcacaaaggaggcgaggttctaagccattcgctcctgctgcttcacaaaaaggaagatggaatttggtccactgatattttaaaggaccagaaagaacccaaaaataagacctttctaagatgcgaggccaagaattattctggacgtttcacctgctggtggctgacgacaatcagtactgatttgacattcagtgtcaaaagcagcagaggctcttctgacccccaaggggtgacgtgcggagctgctacactctctgcagagagagtcagaggggacaacaaggagtatgagtactcagtggagtgccaggaggacagtgcctgcccagctgctgaggagagtctgcccattgaggtcatggtggatgccgttcacaagctcaagtatgaaaactacaccagcagcttcttcatcagggacatcatcaaacctgacccacccaagaacttgcagctgaagccattaaagaattctcggcaggtggaggtcagctgggagtaccctgacacctggagtactccacattcctacttctccctgacattctgcgttcaggtccagggcaagagcaagagagaaaagaaagatagagtcttcacggacaagacctcagccacggtcatctgccgcaaaaatgccagcattagcgtgcgggcccaggaccgctactatagctcatcttggagcgaatgggcatctgtgccctgcagtggtggcggtggaagcggcggtggcggaagcggcggtggcggcagcagaaacctccccgtggccactccagacccaggaatgttcccatgccttcaccactcccaaaacctgctgagggccgtcagcaacatgctccagaaggccagacaaactctagaattttacccttgcacttctgaagagattgatcatgaagatatcacaaaagataaaaccagcacagtggaggcctgtttaccattggaattaaccaagaatgagagttgcctaaattccagagagacctctttcataactaatgggagttgcctggcctccagaaagacctcttttatgatggccctgtgccttagtagtatttatgaagacttgaagatgtaccaggtggagttcaagaccatgaatgcaaagcttctgatggatcctaagaggcagatctttctagatcaaaacatgctggcagttattgatgagctgatgcaggccctgaatttcaacagtgagactgtgccacaaaaatcctcccttgaagaaccggatttttataaaactaaaatcaagctctgcatacttcttcatgctttcagaattcgggcagtgactattgatagagtgatgagctatctgaatgcttcc

SEQ ID NO: 42 - protein, 170 aa, Artificial Sequence
  GAL 3C amino acid construct
MEFGLSWLFLVAILKGVQCSRHHHHHHGAPAGPLIVPYNLPLPGGVVPRMLITILGTVKPNANRIALDFQRGNDVAFHFNPRFNENNRRVIVCNTKLDNNWGREERQSVFPFESGKPFKIQVLVEPDHFKVAVNDAHLLQYNHRVKKLNEISKLGISGDIDLTSASYTMI

SEQ ID NO: 43 - DNA, 510 bp, Artificial Sequence
  GAL 3C nucleic acid construct
atggagtttgggctgagctggctttttcttgtggctattttaaaaggtgtccagtgctctagacatcatcaccatcaccacggcgcccctgctgggccactgattgtgccttataacctgcctttgcctgggggagtggtgcctcgcatgctgataacaattctgggcacggtgaagcccaatgcaaacagaattgctttagatttccaaagagggaatgatgttgccttccactttaacccacgcttcaatgagaacaacaggagagtcattgtttgcaatacaaagctggataataactggggaagggaagaaagacagtcggttttcccatttgaaagtgggaaaccattcaaaatacaagtactggttgaacctgaccacttcaaggttgcagtgaatgatgctcacttgttgcagtacaatcatcgggttaaaaaactcaatgaaatcagcaaactgggaatttctggtgacatagacctcaccagtgcttcatataccatgata